European Patent Specification EP 4 080 219 B1, published November 20, 2024. Title: CONJUGATE. Applicant: DENSO CORPORATION. The sequence listing filed with the application follows.

SEQUENCE LISTING (1 sequence)

SEQ ID NO: 1 - DNA, 51 bp, Artificial Sequence
cagcaccgaccttgtgctttgggagtgctggtccaagggcgttaatggaca